European Patent Application EP 4 261 229 A1, published October 18, 2023. Title: BISPECIFIC ANTIBODY BINDING TO BCMA AND CD3, AND PREPARATION             METHOD THEREFOR AND USE THEREOF. Applicant: EXCYTE BIOPHARMA LTD. The sequence listing filed with the application follows.

SEQUENCE LISTING (52 sequences)

SEQ ID NO: 1 - protein, 13 aa, Artificial Sequence
  Laboratory synthesis
SGSSSNIGGYSVN

SEQ ID NO: 2 - protein, 7 aa, Artificial Sequence
  Laboratory synthesis
RNNQRPS

SEQ ID NO: 3 - protein, 11 aa, Artificial Sequence
  Laboratory synthesis
AAWDDSLIGYV

SEQ ID NO: 4 - protein, 5 aa, Artificial Sequence
  Laboratory synthesis
SYAIS

SEQ ID NO: 5 - protein, 17 aa, Artificial Sequence
  Laboratory synthesis
GIIPIFGTANYAQKFQG

SEQ ID NO: 6 - protein, 6 aa, Artificial Sequence
  Laboratory synthesis
GWYFDL

SEQ ID NO: 7 - protein, 5 aa, Artificial Sequence
  Laboratory synthesis
KSAIM

SEQ ID NO: 8 - protein, 5 aa, Artificial Sequence
  Laboratory synthesis
KSAIQ

SEQ ID NO: 9 - protein, 5 aa, Artificial Sequence
  Laboratory synthesis
KSAIH

SEQ ID NO: 10 - protein, 17 aa, Artificial Sequence
  Laboratory synthesis
GVIPIFGTANYAQKFQG

SEQ ID NO: 11 - protein, 6 aa, Artificial Sequence
  Laboratory synthesis
GWYLDL

SEQ ID NO: 12 - protein, 13 aa, Artificial Sequence
  Laboratory synthesis
SGSSNNIGGYSVN

SEQ ID NO: 13 - protein, 11 aa, Artificial Sequence
  Laboratory synthesis
AAWDDSVIGWL

SEQ ID NO: 14 - protein, 11 aa, Artificial Sequence
  Laboratory synthesis
AAWDDSVIGLL

SEQ ID NO: 15 - protein, 11 aa, Artificial Sequence
  Laboratory synthesis
AAWDDSVIGWV

SEQ ID NO: 16 - protein, 11 aa, Artificial Sequence
  Laboratory synthesis
AAWDDSEIGWL

SEQ ID NO: 17 - protein, 115 aa, Artificial Sequence
  Laboratory synthesis
QVQLQQSGAEVKKPGSSVKVSCKASGGTFSSYAISWVRQAPGQGLEWMGGIIPIFGTANYAQKFQGRVTITADESTSTAYMELSSLRSEDTAVYYCARGWYFDLWGRGTLVTVSS

SEQ ID NO: 18 - protein, 110 aa, Artificial Sequence
  Laboratory synthesis
LPVLTQPPSASGTPGQRVTISCSGSSSNIGGYSVNWYQQFPGTAPKLLIYRNNQRPSGVPDRFSGSKSGASASLAISGLQSEDEADYYCAAWDDSLIGYVFGTGTQLTVL

SEQ ID NO: 19 - protein, 115 aa, Artificial Sequence
  Laboratory synthesis
QVQLQQSGAEVKKPGSSVKVSCKASGGTFSKSAIMWVRQAPGQGLEWMGGVIPIFGTANYAQKFQGRVTITADESTSTAYMELSSLRSEDTAVYYCARGWYLDLWGRGTLVTVSS

SEQ ID NO: 20 - protein, 115 aa, Artificial Sequence
  Laboratory synthesis
QVQLQQSGAEVKKPGSSVKVSCKASGGTFSKSAIQWVRQAPGQGLEWMGGVIPIFGTANYAQKFQGRVTITADESTSTAYMELSSLRSEDTAVYYCARGWYLDLWGRGTLVTVSS

SEQ ID NO: 21 - protein, 115 aa, Artificial Sequence
  Laboratory synthesis
QVQLQQSGAEVKKPGSSVKVSCKASGGTFSKSAIHWVRQAPGQGLEWMGGVIPIFGTANYAQKFQGRVTITADESTSTAYMELSSLRSEDTAVYYCARGWYLDLWGRGTLVTVSS

SEQ ID NO: 22 - protein, 110 aa, Artificial Sequence
  Laboratory synthesis
LPVLTQPPSASGTPGQRVTISCSGSSNNIGGYSVNWYQQFPGTAPKLLIYRNNQRPSGVPDRFSGSKSGASASLAISGLQSEDEADYYCAAWDDSVIGWLFGTGTQLTVL

SEQ ID NO: 23 - protein, 110 aa, Artificial Sequence
  Laboratory synthesis
LPVLTQPPSASGTPGQRVTISCSGSSNNIGGYSVNWYQQFPGTAPKLLIYRNNQRPSGVPDRFSGSKSGASASLAISGLQSEDEADYYCAAWDDSVIGLLFGTGTQLTVL

SEQ ID NO: 24 - protein, 110 aa, Artificial Sequence
  Laboratory synthesis
LPVLTQPPSASGTPGQRVTISCSGSSNNIGGYSVNWYQQFPGTAPKLLIYRNNQRPSGVPDRFSGSKSGASFSLAISGLQFEDEADYYCAAWDDSVIGWVLGTGTQLTVL

SEQ ID NO: 25 - protein, 110 aa, Artificial Sequence
  Laboratory synthesis
LPVLTQPPSASGTPGQRVTISCSGSSSNIGGYSVNWYQQFPGTAPKLLIYRNNQRPSGVPDRFSGSKSGASASLAISGLQSEDVADYYCAAWDDSLIGYVFGTGTQLTVL

SEQ ID NO: 26 - protein, 110 aa, Artificial Sequence
  Laboratory synthesis
LPVLTQPPSASGTPGQRVTISCSGSSNNIGGYSVNWYQQFPGTAPKLLIYRNNQRPSGVPDRFSGSKSGASASLAISGLQSEDEADYYCAAWDDSEIGWLFGTGTQLTVL

SEQ ID NO: 27 - protein, 110 aa, Artificial Sequence
  Laboratory synthesis
LPVLTQPPSASGTPGQRVTISCSGSSNNIGGYSVNWYQQFPGTAPKLLIYRNNQRPSGVPDRFSGSKSGASFSLAISGLQFEDEADYYCARWDDSVIGWVLGTGTQLTVL

SEQ ID NO: 28 - protein, 122 aa, Artificial Sequence
  Laboratory synthesis
EVQLVESGGGLVQPGGSLRLSCAASGYSFTGYTMNWVRQAPGKCLEWVALINPYKGVTTYADSVKGRFTISVDKSKNTAYLQMNSLRAEDTAVYYCARSGYYGDSDWYFDVWGQGTLVTVSS

SEQ ID NO: 29 - protein, 107 aa, Artificial Sequence
  Laboratory synthesis
DIQMTQSPSSLSASVGDRVTITCRASQDIRNYLNWYQQKPGKAPKLLIYYTSRLESGVPSRFSGSGSGTDYTLTISSLQPEDFATYYCQQGNTLPWTFGCGTKVEIK

SEQ ID NO: 30 - protein, 10 aa, Artificial Sequence
  Laboratory synthesis
GGGGSGGGGS

SEQ ID NO: 31 - protein, 244 aa, Artificial Sequence
  Laboratory synthesis
DIQMTQSPSSLSASVGDRVTITCRASQDIRNYLNWYQQKPGKAPKLLIYYTSRLESGVPSRFSGSGSGTDYTLTISSLQPEDFATYYCQQGNTLPWTFGCGTKVEIKGGGGSGGGGSGGGGSEVQLVESGGGLVQPGGSLRLSCAASGYSFTGYTMNWVRQAPGKCLEWVALINPYKGVTTYADSVKGRFTISVDKSKNTAYLQMNSLRAEDTAVYYCARSGYYGDSDWYFDVWGQGTLVTVSS

SEQ ID NO: 32 - protein, 442 aa, Artificial Sequence
  Laboratory synthesis
QVQLQQSGAEVKKPGSSVKVSCKASGGTFSKSAIQWVRQAPGQGLEWMGGVIPIFGTANYAQKFQGRVTITADESTSTAYMELSSLRSEDTAVYYCARGWYLDLWGRGTLVTVSSASTKGPSVFPLAPCSRSTSESTAALGCLVKDYFPEPVTVSWNSGALTSGVHTFPAVLQSSGLYSLSSVVTVPSSSLGTKTYTCNVDHKPSNTKVDKRVESKYGPPCPPCPAPEFLGGPSVFLFPPKPKDTLMISRTPEVTCVVVDVSQEDPEVQFNWYVDGVEVHNAKTKPREEQFNSTYRVVSVLTVLHQDWLNGKEYKCKVSNKGLPSSIEKTISKAKGQPREPQVYTLPPSQEEMTKNQVSLTCLVKGFYPSDIAVEWESNGQPENNYKTTPPVLDSDGSFFLYSRLTVDKSRWQEGNVFSCSVMHEALHNHYTQKSLSLSLGK

SEQ ID NO: 33 - protein, 216 aa, Artificial Sequence
  Laboratory synthesis
LPVLTQPPSASGTPGQRVTISCSGSSNNIGGYSVNWYQQFPGTAPKLLIYRNNQRPSGVPDRFSGSKSGASASLAISGLQSEDEADYYCAAWDDSVIGWLFGTGTQLTVLGQPKAAPSVTLFPPSSEELQANKATLVCLISDFYPGAVTVAWKADSSPVKAGVETTTPSKQSNNKYAASSYLSLTPEQWKSHRSYSCQVTHEGSTVEKTVAPTECS

SEQ ID NO: 34 - protein, 696 aa, Artificial Sequence
  Laboratory synthesis
DIQMTQSPSSLSASVGDRVTITCRASQDIRNYLNWYQQKPGKAPKLLIYYTSRLESGVPSRFSGSGSGTDYTLTISSLQPEDFATYYCQQGNTLPWTFGCGTKVEIKGGGGSGGGGSGGGGSEVQLVESGGGLVQPGGSLRLSCAASGYSFTGYTMNWVRQAPGKCLEWVALINPYKGVTTYADSVKGRFTISVDKSKNTAYLQMNSLRAEDTAVYYCARSGYYGDSDWYFDVWGQGTLVTVSSGGGGSGGGGSQVQLQQSGAEVKKPGSSVKVSCKASGGTFSSYAISWVRQAPGQGLEWMGGIIPIFGTANYAQKFQGRVTITADESTSTAYMELSSLRSEDTAVYYCARGWYFDLWGRGTLVTVSSASTKGPSVFPLAPCSRSTSESTAALGCLVKDYFPEPVTVSWNSGALTSGVHTFPAVLQSSGLYSLSSVVTVPSSSLGTKTYTCNVDHKPSNTKVDKRVESKYGPPCPPCPAPEFLGGPSVFLFPPKPKDTLMISRTPEVTCVVVDVSQEDPEVQFNWYVDGVEVHNAKTKPREEQFNSTYRVVSVLTVLHQDWLNGKEYKCKVSNKGLPSSIEKTISKAKGQPREPQVYTLPPSQEEMTKNQVSLTCLVKGFYPSDIAVEWESNGQPENNYKTTPPVLDSDGSFFLYSRLTVDKSRWQEGNVFSCSVMHEALHNHYTQKSLSLSLGK

SEQ ID NO: 35 - protein, 696 aa, Artificial Sequence
  Laboratory synthesis
QVQLQQSGAEVKKPGSSVKVSCKASGGTFSKSAIQWVRQAPGQGLEWMGGVIPIFGTANYAQKFQGRVTITADESTSTAYMELSSLRSEDTAVYYCARGWYLDLWGRGTLVTVSSASTKGPSVFPLAPCSRSTSESTAALGCLVKDYFPEPVTVSWNSGALTSGVHTFPAVLQSSGLYSLSSVVTVPSSSLGTKTYTCNVDHKPSNTKVDKRVESKYGPPCPPCPAPEFLGGPSVFLFPPKPKDTLMISRTPEVTCVVVDVSQEDPEVQFNWYVDGVEVHNAKTKPREEQFNSTYRVVSVLTVLHQDWLNGKEYKCKVSNKGLPSSIEKTISKAKGQPREPQVYTLPPSQEEMTKNQVSLTCLVKGFYPSDIAVEWESNGQPENNYKTTPPVLDSDGSFFLYSRLTVDKSRWQEGNVFSCSVMHEALHNHYTQKSLSLSLGKGGGGSGGGGSDIQMTQSPSSLSASVGDRVTITCRASQDIRNYLNWYQQKPGKAPKLLIYYTSRLESGVPSRFSGSGSGTDYTLTISSLQPEDFATYYCQQGNTLPWTFGCGTKVEIKGGGGSGGGGSGGGGSEVQLVESGGGLVQPGGSLRLSCAASGYSFTGYTMNWVRQAPGKCLEWVALINPYKGVTTYADSVKGRFTISVDKSKNTAYLQMNSLRAEDTAVYYCARSGYYGDSDWYFDVWGQGTLVTVSS

SEQ ID NO: 36 - protein, 246 aa, Artificial Sequence
  Laboratory synthesis
QVQLQQSGAEVKKPGSSVKVSCKASGGTFSSYAISWVRQAPGQGLEWMGGIIPIFGTANYAQKFQGRVTITADESTSTAYMELSSLRSEDTAVYYCARGWYFDLWGRGTLVTVSSASTGGSSRSSSSGGGGSGGGGLPVLTQPPSASGTPGQRVTISCSGSSSNIGGYSVNWYQQFPGTAPKLLIYRNNQRPSGVPDRFSGSKSGASASLAISGLQSEDEADYYCAAWDDSLIGYVFGTGTQLTVL

SEQ ID NO: 37 - protein, 246 aa, Artificial Sequence
  Laboratory synthesis
QVQLQQSGAEVKKPGSSVKVSCKASGGTFSKSAIQWVRQAPGQGLEWMGGVIPIFGTANYAQKFQGRVTITADESTSTAYMELSSLRSEDTAVYYCARGWYLDLWGRGTLVTVSSASTGGSSRSSSSGGGGSGGGGLPVLTQPPSASGTPGQRVTISCSGSSNNIGGYSVNWYQQFPGTAPKLLIYRNNQRPSGVPDRFSGSKSGASASLAISGLQSEDEADYYCAAWDDSVIGWLFGTGTQLTVL

SEQ ID NO: 38 - protein, 246 aa, Artificial Sequence
  Laboratory synthesis
QVQLQQSGAEVKKPGSSVKVSCKASGGTFSKSAIMWVRQAPGQGLEWMGGVIPIFGTANYAQKFQGRVTITADESTSTAYMELSSLRSEDTAVYYCARGWYLDLWGRGTLVTVSSASTGGSSRSSSSGGGGSGGGGLPVLTQPPSASGTPGQRVTISCSGSSNNIGGYSVNWYQQFPGTAPKLLIYRNNQRPSGVPDRFSGSKSGASFSLAISGLQFEDEADYYCARWDDSVIGWVLGTGTQLTVL

SEQ ID NO: 39 - protein, 246 aa, Artificial Sequence
  Laboratory synthesis
QVQLQQSGAEVKKPGSSVKVSCKASGGTFSKSAIHWVRQAPGQGLEWMGGVIPIFGTANYAQKFQGRVTITADESTSTAYMELSSLRSEDTAVYYCARGWYLDLWGRGTLVTVSSASTGGSSRSSSSGGGGSGGGGLPVLTQPPSASGTPGQRVTISCSGSSSNIGGYSVNWYQQFPGTAPKLLIYRNNQRPSGVPDRFSGSKSGASASLAISGLQSEDVADYYCAAWDDSLIGYVFGTGTQLTVL

SEQ ID NO: 40 - protein, 246 aa, Artificial Sequence
  Laboratory synthesis
QVQLQQSGAEVKKPGSSVKVSCKASGGTFSKSAIQWVRQAPGQGLEWMGGVIPIFGTANYAQKFQGRVTITADESTSTAYMELSSLRSEDTAVYYCARGWYLDLWGRGTLVTVSSASTGGSSRSSSSGGGGSGGGGLPVLTQPPSASGTPGQRVTISCSGSSNNIGGYSVNWYQQFPGTAPKLLIYRNNQRPSGVPDRFSGSKSGASASLAISGLQSEDEADYYCAAWDDSEIGWLFGTGTQLTVL

SEQ ID NO: 41 - protein, 696 aa, Artificial Sequence
  Laboratory synthesis
QVQLQQSGAEVKKPGSSVKVSCKASGGTFSSYAISWVRQAPGQGLEWMGGIIPIFGTANYAQKFQGRVTITADESTSTAYMELSSLRSEDTAVYYCARGWYFDLWGRGTLVTVSSASTKGPSVFPLAPCSRSTSESTAALGCLVKDYFPEPVTVSWNSGALTSGVHTFPAVLQSSGLYSLSSVVTVPSSSLGTKTYTCNVDHKPSNTKVDKRVESKYGPPCPPCPAPEFLGGPSVFLFPPKPKDTLMISRTPEVTCVVVDVSQEDPEVQFNWYVDGVEVHNAKTKPREEQFNSTYRVVSVLTVLHQDWLNGKEYKCKVSNKGLPSSIEKTISKAKGQPREPQVYTLPPSQEEMTKNQVSLTCLVKGFYPSDIAVEWESNGQPENNYKTTPPVLDSDGSFFLYSRLTVDKSRWQEGNVFSCSVMHEALHNHYTQKSLSLSLGKGGGGSGGGGSDIQMTQSPSSLSASVGDRVTITCRASQDIRNYLNWYQQKPGKAPKLLIYYTSRLESGVPSRFSGSGSGTDYTLTISSLQPEDFATYYCQQGNTLPWTFGCGTKVEIKGGGGSGGGGSGGGGSEVQLVESGGGLVQPGGSLRLSCAASGYSFTGYTMNWVRQAPGKCLEWVALINPYKGVTTYADSVKGRFTISVDKSKNTAYLQMNSLRAEDTAVYYCARSGYYGDSDWYFDVWGQGTLVTVSS

SEQ ID NO: 42 - protein, 216 aa, Artificial Sequence
  Laboratory synthesis
LPVLTQPPSASGTPGQRVTISCSGSSSNIGGYSVNWYQQFPGTAPKLLIYRNNQRPSGVPDRFSGSKSGASASLAISGLQSEDEADYYCAAWDDSLIGYVFGTGTQLTVLGQPKAAPSVTLFPPSSEELQANKATLVCLISDFYPGAVTVAWKADSSPVKAGVETTTPSKQSNNKYAASSYLSLTPEQWKSHRSYSCQVTHEGSTVEKTVAPTECS

SEQ ID NO: 43 - protein, 696 aa, Artificial Sequence
  Laboratory synthesis
QVQLQQSGAEVKKPGSSVKVSCKASGGTFSKSAIMWVRQAPGQGLEWMGGVIPIFGTANYAQKFQGRVTITADESTSTAYMELSSLRSEDTAVYYCARGWYLDLWGRGTLVTVSSASTKGPSVFPLAPCSRSTSESTAALGCLVKDYFPEPVTVSWNSGALTSGVHTFPAVLQSSGLYSLSSVVTVPSSSLGTKTYTCNVDHKPSNTKVDKRVESKYGPPCPPCPAPEFLGGPSVFLFPPKPKDTLMISRTPEVTCVVVDVSQEDPEVQFNWYVDGVEVHNAKTKPREEQFNSTYRVVSVLTVLHQDWLNGKEYKCKVSNKGLPSSIEKTISKAKGQPREPQVYTLPPSQEEMTKNQVSLTCLVKGFYPSDIAVEWESNGQPENNYKTTPPVLDSDGSFFLYSRLTVDKSRWQEGNVFSCSVMHEALHNHYTQKSLSLSLGKGGGGSGGGGSDIQMTQSPSSLSASVGDRVTITCRASQDIRNYLNWYQQKPGKAPKLLIYYTSRLESGVPSRFSGSGSGTDYTLTISSLQPEDFATYYCQQGNTLPWTFGCGTKVEIKGGGGSGGGGSGGGGSEVQLVESGGGLVQPGGSLRLSCAASGYSFTGYTMNWVRQAPGKCLEWVALINPYKGVTTYADSVKGRFTISVDKSKNTAYLQMNSLRAEDTAVYYCARSGYYGDSDWYFDVWGQGTLVTVSS

SEQ ID NO: 44 - protein, 216 aa, Artificial Sequence
  Laboratory synthesis
LPVLTQPPSASGTPGQRVTISCSGSSNNIGGYSVNWYQQFPGTAPKLLIYRNNQRPSGVPDRFSGSKSGASFSLAISGLQFEDEADYYCARWDDSVIGWVLGTGTQLTVLGQPKAAPSVTLFPPSSEELQANKATLVCLISDFYPGAVTVAWKADSSPVKAGVETTTPSKQSNNKYAASSYLSLTPEQWKSHRSYSCQVTHEGSTVEKTVAPTECS

SEQ ID NO: 45 - protein, 696 aa, Artificial Sequence
  Laboratory synthesis
QVQLQQSGAEVKKPGSSVKVSCKASGGTFSKSAIHWVRQAPGQGLEWMGGVIPIFGTANYAQKFQGRVTITADESTSTAYMELSSLRSEDTAVYYCARGWYLDLWGRGTLVTVSSASTKGPSVFPLAPCSRSTSESTAALGCLVKDYFPEPVTVSWNSGALTSGVHTFPAVLQSSGLYSLSSVVTVPSSSLGTKTYTCNVDHKPSNTKVDKRVESKYGPPCPPCPAPEFLGGPSVFLFPPKPKDTLMISRTPEVTCVVVDVSQEDPEVQFNWYVDGVEVHNAKTKPREEQFNSTYRVVSVLTVLHQDWLNGKEYKCKVSNKGLPSSIEKTISKAKGQPREPQVYTLPPSQEEMTKNQVSLTCLVKGFYPSDIAVEWESNGQPENNYKTTPPVLDSDGSFFLYSRLTVDKSRWQEGNVFSCSVMHEALHNHYTQKSLSLSLGKGGGGSGGGGSDIQMTQSPSSLSASVGDRVTITCRASQDIRNYLNWYQQKPGKAPKLLIYYTSRLESGVPSRFSGSGSGTDYTLTISSLQPEDFATYYCQQGNTLPWTFGCGTKVEIKGGGGSGGGGSGGGGSEVQLVESGGGLVQPGGSLRLSCAASGYSFTGYTMNWVRQAPGKCLEWVALINPYKGVTTYADSVKGRFTISVDKSKNTAYLQMNSLRAEDTAVYYCARSGYYGDSDWYFDVWGQGTLVTVSS

SEQ ID NO: 46 - protein, 216 aa, Artificial Sequence
  Laboratory synthesis
LPVLTQPPSASGTPGQRVTISCSGSSSNIGGYSVNWYQQFPGTAPKLLIYRNNQRPSGVPDRFSGSKSGASASLAISGLQSEDVADYYCAAWDDSLIGYVFGTGTQLTVLGQPKAAPSVTLFPPSSEELQANKATLVCLISDFYPGAVTVAWKADSSPVKAGVETTTPSKQSNNKYAASSYLSLTPEQWKSHRSYSCQVTHEGSTVEKTVAPTECS

SEQ ID NO: 47 - protein, 696 aa, Artificial Sequence; identical to SEQ ID NO: 35
  Laboratory synthesis

SEQ ID NO: 48 - protein, 216 aa, Artificial Sequence
  Laboratory synthesis
LPVLTQPPSASGTPGQRVTISCSGSSNNIGGYSVNWYQQFPGTAPKLLIYRNNQRPSGVPDRFSGSKSGASASLAISGLQSEDEADYYCAAWDDSEIGWLFGTGTQLTVLGQPKAAPSVTLFPPSSEELQANKATLVCLISDFYPGAVTVAWKADSSPVKAGVETTTPSKQSNNKYAASSYLSLTPEQWKSHRSYSCQVTHEGSTVEKTVAPTECS

SEQ ID NO: 49 - protein, 442 aa, Artificial Sequence
  Laboratory synthesis
QVQLQQSGAEVKKPGSSVKVSCKASGGTFSSYAISWVRQAPGQGLEWMGGIIPIFGTANYAQKFQGRVTITADESTSTAYMELSSLRSEDTAVYYCARGWYFDLWGRGTLVTVSSASTKGPSVFPLAPCSRSTSESTAALGCLVKDYFPEPVTVSWNSGALTSGVHTFPAVLQSSGLYSLSSVVTVPSSSLGTKTYTCNVDHKPSNTKVDKRVESKYGPPCPPCPAPEFLGGPSVFLFPPKPKDTLMISRTPEVTCVVVDVSQEDPEVQFNWYVDGVEVHNAKTKPREEQFNSTYRVVSVLTVLHQDWLNGKEYKCKVSNKGLPSSIEKTISKAKGQPREPQVYTLPPSQEEMTKNQVSLTCLVKGFYPSDIAVEWESNGQPENNYKTTPPVLDSDGSFFLYSRLTVDKSRWQEGNVFSCSVMHEALHNHYTQKSLSLSLGK

SEQ ID NO: 50 - protein, 442 aa, Artificial Sequence
  Laboratory synthesis
QVQLQQSGAEVKKPGSSVKVSCKASGGTFSKSAIMWVRQAPGQGLEWMGGVIPIFGTANYAQKFQGRVTITADESTSTAYMELSSLRSEDTAVYYCARGWYLDLWGRGTLVTVSSASTKGPSVFPLAPCSRSTSESTAALGCLVKDYFPEPVTVSWNSGALTSGVHTFPAVLQSSGLYSLSSVVTVPSSSLGTKTYTCNVDHKPSNTKVDKRVESKYGPPCPPCPAPEFLGGPSVFLFPPKPKDTLMISRTPEVTCVVVDVSQEDPEVQFNWYVDGVEVHNAKTKPREEQFNSTYRVVSVLTVLHQDWLNGKEYKCKVSNKGLPSSIEKTISKAKGQPREPQVYTLPPSQEEMTKNQVSLTCLVKGFYPSDIAVEWESNGQPENNYKTTPPVLDSDGSFFLYSRLTVDKSRWQEGNVFSCSVMHEALHNHYTQKSLSLSLGK

SEQ ID NO: 51 - protein, 442 aa, Artificial Sequence
  Laboratory synthesis
QVQLQQSGAEVKKPGSSVKVSCKASGGTFSKSAIHWVRQAPGQGLEWMGGVIPIFGTANYAQKFQGRVTITADESTSTAYMELSSLRSEDTAVYYCARGWYLDLWGRGTLVTVSSASTKGPSVFPLAPCSRSTSESTAALGCLVKDYFPEPVTVSWNSGALTSGVHTFPAVLQSSGLYSLSSVVTVPSSSLGTKTYTCNVDHKPSNTKVDKRVESKYGPPCPPCPAPEFLGGPSVFLFPPKPKDTLMISRTPEVTCVVVDVSQEDPEVQFNWYVDGVEVHNAKTKPREEQFNSTYRVVSVLTVLHQDWLNGKEYKCKVSNKGLPSSIEKTISKAKGQPREPQVYTLPPSQEEMTKNQVSLTCLVKGFYPSDIAVEWESNGQPENNYKTTPPVLDSDGSFFLYSRLTVDKSRWQEGNVFSCSVMHEALHNHYTQKSLSLSLGK

SEQ ID NO: 52 - protein, 442 aa, Artificial Sequence; identical to SEQ ID NO: 32
  Laboratory synthesis